European Patent Specification EP 3 318 269 B1, published March 13, 2024. Title: METHODS FOR TREATMENT OF NEPHROTIC SYNDROME AND RELATED CONDITIONS. Applicant: The UAB Research Foundation Chugh, Sumant  S. The sequence listing filed with the application follows.

SEQUENCE LISTING (22 sequences)

SEQ ID NO: 1 - protein, 406 aa, Homo sapiens
MSGAPTAGAALMLCAATAVLLSAQGGPVQSKSPRFASWDEMNVLAHGLLQLGQGLREHAERTRSQLSALERRLSACGSACQGTEGSTDLPLAPESRVDPEVLHSLQTQLKAQNSRIQQLFHKVAQQQRHLEKQHLRIQHLQSQFGLLDHKHLDHEVAKPARRKRLPEMAQPVDPAHNVSRLHRLPRDCQELFQVGERQSGLFEIQPQGSPPFLVNCKMTSDGGWTVIQRRHDGSVDFNRPWEAYKAGFGDPHGEFWLGLEKVHSITGDRNSRLAVQLRDWDGNAELLQFSVHLGGEDTAYSLQLTAPVAGQLGATTVPPSGLSVPFSTWDQDHDLRRDKNCAKSLSGGWWFGTCSHSNLNGQYFRSIPQQRQKLKKGIFWKTWRGRYYPLQATTMLIQPMAAEAAS

SEQ ID NO: 2 - DNA, 1967 bp, Homo sapiens
ataaaaaccgtcctcgggcgcggcggggagaagccgagctgagcggatcctcacacgactgtgatccgattctttccagcggcttctgcaaccaagcgggtcttacccccggtcctccgcgtctccagtcctcgcacctggaaccccaacgtccccgagagtccccgaatccccgctcccaggctacctaagaggatgagcggtgctccgacggccggggcagccctgatgctctgcgccgccaccgccgtgctactgagcgctcagggcggacccgtgcagtccaagtcgccgcgctttgcgtcctgggacgagatgaatgtcctggcgcacggactcctgcagctcggccaggggctgcgcgaacacgcggagcgcacccgcagtcagctgagcgcgctggagcggcgcctgagcgcgtgcgggtccgcctgtcagggaaccgaggggtccaccgacctcccgttagcccctgagagccgggtggaccctgaggtccttcacagcctgcagacacaactcaaggctcagaacagcaggatccagcaactcttccacaaggtggcccagcagcagcggcacctggagaagcagcacctgcgaattcagcatctgcaaagccagtttggcctcctggaccacaagcacctagaccatgaggtggccaagcctgcccgaagaaagaggctgcccgagatggcccagccagttgacccggctcacaatgtcagccgcctgcaccggctgcccagggattgccaggagctgttccaggttggggagaggcagagtggactatttgaaatccagcctcaggggtctccgccatttttggtgaactgcaagatgacctcagatggaggctggacagtaattcagaggcgccacgatggctcagtggacttcaaccggccctgggaagcctacaaggcggggtttggggatccccacggcgagttctggctgggtctggagaaggtgcatagcatcacgggggaccgcaacagccgcctggccgtgcagctgcgggactgggatggcaacgccgagttgctgcagttctccgtgcacctgggtggcgaggacacggcctatagcctgcagctcactgcacccgtggccggccagctgggcgccaccaccgtcccacccagcggcctctccgtacccttctccacttgggaccaggatcacgacctccgcagggacaagaactgcgccaagagcctctctggaggctggtggtttggcacctgcagccattccaacctcaacggccagtacttccgctccatcccacagcagcggcagaagcttaagaagggaatcttctggaagacctggcggggccgctactacccgctgcaggccaccaccatgttgatccagcccatggcagcagaggcagcctcctagcgtcctggctgggcctggtcccaggcccacgaaagacggtgactcttggctctgcccgaggatgtggccgttccctgcctgggcaggggctccaaggaggggccatctggaaacttgtggacagagaagaagaccacgactggagaagccccctttctgagtgcaggggggctgcatgcgttgcctcctgagatcgaggctgcaggatatgctcagactctagaggcgtggaccaaggggcatggagcttcactccttgctggccagggagttggggactcagagggaccacttggggccagccagactggcctcaatggcggactcagtcacattgactgacggggaccagggcttgtgtgggtcgagagcgccctcatggtgctggtgctgttgtgtgtaggtcccctggggacacaagcaggcgccaatggtatctgggcggagctcacagagttcttggaataaaagcaacctcagaacacttaaaaaaaaaaaaaaaaaaaaaaaaaaaaaaaaaaaaaaaaaaaaaaaaaaaaaaaaaaaaaaaa

SEQ ID NO: 3 - protein, 368 aa, Homo sapiens
MSGAPTAGAALMLCAATAVLLSAQGGPVQSKSPRFASWDEMNVLAHGLLQLGQGLREHAERTRSQLSALERRLSACGSACQGTEGSTDLPLAPESRVDPEVLHSLQTQLKAQNSRIQQLFHKVAQQQRHLEKQHLRIQHLQSQFGLLDHKHLDHEVAKPARRKRLPEMAQPVDPAHNVSRLHHGGWTVIQRRHDGSVDFNRPWEAYKAGFGDPHGEFWLGLEKVHSITGDRNSRLAVQLRDWDGNAELLQFSVHLGGEDTAYSLQLTAPVAGQLGATTVPPSGLSVPFSTWDQDHDLRRDKNCAKSLSGGWWFGTCSHSNLNGQYFRSIPQQRQKLKKGIFWKTWRGRYYPLQATTMLIQPMAAEAAS

SEQ ID NO: 4 - DNA, 1853 bp, Homo sapiens
ataaaaaccgtcctcgggcgcggcggggagaagccgagctgagcggatcctcacacgactgtgatccgattctttccagcggcttctgcaaccaagcgggtcttacccccggtcctccgcgtctccagtcctcgcacctggaaccccaacgtccccgagagtccccgaatccccgctcccaggctacctaagaggatgagcggtgctccgacggccggggcagccctgatgctctgcgccgccaccgccgtgctactgagcgctcagggcggacccgtgcagtccaagtcgccgcgctttgcgtcctgggacgagatgaatgtcctggcgcacggactcctgcagctcggccaggggctgcgcgaacacgcggagcgcacccgcagtcagctgagcgcgctggagcggcgcctgagcgcgtgcgggtccgcctgtcagggaaccgaggggtccaccgacctcccgttagcccctgagagccgggtggaccctgaggtccttcacagcctgcagacacaactcaaggctcagaacagcaggatccagcaactcttccacaaggtggcccagcagcagcggcacctggagaagcagcacctgcgaattcagcatctgcaaagccagtttggcctcctggaccacaagcacctagaccatgaggtggccaagcctgcccgaagaaagaggctgcccgagatggcccagccagttgacccggctcacaatgtcagccgcctgcaccatggaggctggacagtaattcagaggcgccacgatggctcagtggacttcaaccggccctgggaagcctacaaggcggggtttggggatccccacggcgagttctggctgggtctggagaaggtgcatagcatcacgggggaccgcaacagccgcctggccgtgcagctgcgggactgggatggcaacgccgagttgctgcagttctccgtgcacctgggtggcgaggacacggcctatagcctgcagctcactgcacccgtggccggccagctgggcgccaccaccgtcccacccagcggcctctccgtacccttctccacttgggaccaggatcacgacctccgcagggacaagaactgcgccaagagcctctctggaggctggtggtttggcacctgcagccattccaacctcaacggccagtacttccgctccatcccacagcagcggcagaagcttaagaagggaatcttctggaagacctggcggggccgctactacccgctgcaggccaccaccatgttgatccagcccatggcagcagaggcagcctcctagcgtcctggctgggcctggtcccaggcccacgaaagacggtgactcttggctctgcccgaggatgtggccgttccctgcctgggcaggggctccaaggaggggccatctggaaacttgtggacagagaagaagaccacgactggagaagccccctttctgagtgcaggggggctgcatgcgttgcctcctgagatcgaggctgcaggatatgctcagactctagaggcgtggaccaaggggcatggagcttcactccttgctggccagggagttggggactcagagggaccacttggggccagccagactggcctcaatggcggactcagtcacattgactgacggggaccagggcttgtgtgggtcgagagcgccctcatggtgctggtgctgttgtgtgtaggtcccctggggacacaagcaggcgccaatggtatctgggcggagctcacagagttcttggaataaaagcaacctcagaacacttaaaaaaaaaaaaaaaaaaaaaaaaaaaaaaaaaaaaaaaaaaaaaaaaaaaaaaaaaaaaaaaa

SEQ ID NO: 5 - protein, 405 aa, Rattus norvegicus
MRCAPTAGAALVLCAATAGLLSAQGRPAQPEPPRFASWDEMNLLAHGLLQLGHGLREHVERTRGQLGALERRMAACGNACQGPKGTDPKDRVPEGQAPETLQSLQTQLKAQNSKIQQLFQKVAQQQRYLSKQNLRIQNLQSQIDLLTPTHLDNGVDKTSRGKRLPKMAQLIGLTPNATRLHRPPRDCQELFQEGERHSGLFQIQPLGSPPFLVNCEMTSDGGWTVIQRRLNGSVDFNQSWEAYKDGFGDPQGEFWLGLEKMHSITGDRGSQLAVQLQDWDGNAKLLQFPIHLGGEDTAYSLQLTEPTANELGATNVSPNGLSLPFSTWDQDHDLRGDLNCAKSLSGGWWFGTCSHSNLNGQYFHSIPRQRQQRKKGIFWKTWKGRYYPLQATTLLIQPMEATAAS

SEQ ID NO: 6 - DNA, 1218 bp, Rattus norvegicus
atgcgctgcgctccgaccgcaggcgctgctctagtgctatgcgcagctactgcggggctgctgagcgcgcaagggcgccctgcacagccggagccgccgcgcttcgcatcctgggatgaaatgaacttgctggctcacgggctgctgcagctcggtcacgggctgcgggaacacgtggagcgcacccgtggacagctgggcgcgctggaacgccgcatggctgcctgcggtaacgcttgtcaggggcccaaggggacagacccgaaggatagagtccccgaaggccaggctcctgagactctgcagagtttacagactcaactcaaggctcagaacagcaagatccagcaactgttccagaaggtagcccagcagcagagatacctatcaaagcagaatctgagaatacagaatcttcagagccagattgacctcttgacccccacacacctagacaatggggtagacaagacttcgaggggaaagaggcttcccaagatggcccagctcattggcttgactcccaacgccacccgcttacacaggcctccccgggactgccaggaactctttcaagaaggggagcggcacagtggacttttccagatccagcctctgggatctccaccatttttggtcaactgtgagatgacttcagatggaggctggacggtgattcagagacgcctgaacggctctgtggacttcaatcagtcttgggaagcctacaaagatggcttcggagatccccaaggcgagttctggctgggcctagagaagatgcacagcatcacaggggaccgaggaagccagttggctgtgcagctccaggactgggatggcaatgccaaattgctccaatttcctatccatttggggggtgaggacacagcctacagcctgcagctcaccgagcccacggccaatgagctgggtgccaccaatgtttcccccaatggcctttccctgcccttctctacctgggaccaagaccacgacctccgaggggaccttaactgtgccaagagcctctctggtggctggtggtttggcacctgcagccattccaatctaaatggacaatacttccactctattccacggcaacggcagcagcgtaaaaaggggatcttctggaaaacatggaagggccgctactatccactacaggctaccaccctgttgatccagcccatggaggctacagcagcctcttag

SEQ ID NO: 7 - protein, 410 aa, Mus musculus
MRCAPTAGAALVLCAATAGLLSAQGRPAQPEPPRFASWDEMNLLAHGLLQLGHGLREHVERTRGQLGALERRMAACGNACQGPKGKDAPFKDSEDRVPEGQTPETLQSLQTQLKAQNSKIQQLFQKVAQQQRYLSKQNLRIQNLQSQIDLLAPTHLDNGVDKTSRGKRLPKMTQLIGLTPNATHLHRPPRDCQELFQEGERHSGLFQIQPLGSPPFLVNCEMTSDGGWTVIQRRLNGSVDFNQSWEAYKDGFGDPQGEFWLGLEKMHSITGNRGSQLAVQLQDWDGNAKLLQFPIHLGGEDTAYSLQLTEPTANELGATNVSPNGLSLPFSTWDQDHDLRGDLNCAKSLSGGWWFGTCSHSNLNGQYFHSIPRQRQERKKGIFWKTWKGRYYPLQATTLLIQPMEATAAS

SEQ ID NO: 8 - DNA, 1869 bp, Mus musculus
acgggctccagatcttcttctgcaccagagcaagtctaagtctgagccggctcccccagaactccagctgctgggtcttgaactcctgcgttccggagtcctagcgttgctgcacccaaggccacccccagaatcatgcgctgcgctccgacagcaggcgctgccctggtgctatgcgcggctactgcggggcttttgagcgcgcaagggcgccctgcacagccagagccaccgcgctttgcatcctgggacgagatgaacttgctggctcacgggctgctacagctcggccatgggctgcgcgaacacgtggagcgcacccgtgggcagctgggcgcgctggagcgccgcatggctgcctgtggtaacgcttgtcaggggcccaagggaaaagatgcacccttcaaagactccgaggatagagtccctgaaggccagactcctgagactctgcagagtttgcagactcagctcaaggctcaaaacagcaagatccagcaattgttccagaaggtggcccagcagcagagatacctatcaaagcagaatctgagaatacagaatcttcagagccagatagacctcttggcccccacgcacctagacaatggagtagacaagacttcgaggggaaagaggcttcccaagatgacccagctcattggcttgactcccaacgccacccacttacacaggccgccccgggactgccaggaactcttccaagaaggggagaggcacagtggacttttccagatccagcctctggggtctccaccatttttggtcaactgtgagatgacttcagatggaggctggacagtgattcagagacgcctgaacggctctgtggacttcaaccagtcctgggaagcctacaaggatggcttcggagatccccaaggcgagttctggctgggcctggaaaagatgcacagcatcacagggaaccgaggaagccaattggctgtgcagctccaggactgggatggcaatgccaaattgctccaatttcccatccatttggggggtgaggacacagcctacagcctgcagctcactgagcccacggccaatgagctgggtgccaccaatgtttcccccaatggcctttccctgcccttctctacttgggaccaagaccatgacctccgtggggaccttaactgtgccaagagcctctctggtggctggtggtttggtacctgtagccattccaatctcaatggacaatacttccactctatcccacggcaacggcaggagcgtaaaaagggtatcttctggaaaacatggaagggccgctactatcctctgcaggctaccaccctgctgatccagcccatggaggctacagcagcctcttagcctcctcactggagcctggttccaggcctaagaagacagtgactttggttgtggccctgagatttggccattctctgctgggggcaggagctctaagtagggctatctgcgtcttgtggacaaagaagaagcccgtaactggagagactggaggaccccttttccgtgttggggtctgcaagcattgttgtctgaaacagtcagagcaacaggaaacaaatggcccagatccagaaaacatgggctcgaggggcactgaatatcacttctcgcctaccagagaagttggggatgcagagggaccactacagtccaactagctgggcccttaatggcggactcagtcatattgactgactggagacagggtgccaggagccctggatacactcatggtgctgttgtaggtgctgtggatgcacaggtgctaactgtggttcccaggcacaactcacagcattcttacaataaaaacaacctcagaacaaaaaaaaaaaaaaa

SEQ ID NO: 9 - protein, 406 aa, Homo sapiens
  MISC_FEATURE (39)..(39): x = A, K, E or D
  MISC_FEATURE (40)..(40): x = A, K, E or D
  MISC_FEATURE (76)..(76): x = A or S
  MISC_FEATURE (80)..(80): x = A or S
  MISC_FEATURE (161)..(161): x = D, R, K, G, A, V or S
  MISC_FEATURE (162)..(162): x = D, R, K, G, A, V or S
  MISC_FEATURE (163)..(163): x = D, R, K, G, A, V or S
  MISC_FEATURE (164)..(164): x = D, R, K, G, A, V or S
  misc_feature (221)..(221): Xaa can be any naturally occurring amino acid
MSGAPTAGAALMLCAATAVLLSAQGGPVQSKSPRFASWXXMNVLAHGLLQLGQGLREHAERTRSQLSALERRLSAXGSAXQGTEGSTDLPLAPESRVDPEVLHSLQTQLKAQNSRIQQLFHKVAQQQRHLEKQHLRIQHLQSQFGLLDHKHLDHEVAKPAXXXXLPEMAQPVDPAHNVSRLHRLPRDCQELFQVGERQSGLFEIQPQGSPPFLVNCKMTSXGGWTVIQRRHDGSVDFNRPWEAYKAGFGDPHGEFWLGLEKVHSITGDRNSRLAVQLRDWDGNAELLQFSVHLGGEDTAYSLQLTAPVAGQLGATTVPPSGLSVPFSTWDQDHDLRRDKNCAKSLSGGWWFGTCSHSNLNGQYFRSIPQQRQKLKKGIFWKTWRGRYYPLQATTMLIQPMAAEAAS

SEQ ID NO: 10 - protein, 368 aa, Homo sapiens
  MISC_FEATURE (39)..(39): x = A, K, D or E
  MISC_FEATURE (40)..(40): x = A, K, D or E
  MISC_FEATURE (76)..(76): x = A or C
  MISC_FEATURE (80)..(80): x = A or C
  MISC_FEATURE (161)..(161): x = D, R, K, G, A, V or S
  MISC_FEATURE (162)..(162): x = D, R, K, G, A, V or S
  MISC_FEATURE (163)..(163): x = D, R, K, G, A, V or S
  MISC_FEATURE (164)..(164): x = D, R, K, G, A, V or S
MSGAPTAGAALMLCAATAVLLSAQGGPVQSKSPRFASWXXMNVLAHGLLQLGQGLREHAERTRSQLSALERRLSAXGSAXQGTEGSTDLPLAPESRVDPEVLHSLQTQLKAQNSRIQQLFHKVAQQQRHLEKQHLRIQHLQSQFGLLDHKHLDHEVAKPAXXXXLPEMAQPVDPAHNVSRLHHGGWTVIQRRHDGSVDFNRPWEAYKAGFGDPHGEFWLGLEKVHSITGDRNSRLAVQLRDWDGNAELLQFSVHLGGEDTAYSLQLTAPVAGQLGATTVPPSGLSVPFSTWDQDHDLRRDKNCAKSLSGGWWFGTCSHSNLNGQYFRSIPQQRQKLKKGIFWKTWRGRYYPLQATTMLIQPMAAEAAS

SEQ ID NO: 11 - DNA, 22 bp, Homo sapiens
tctgggatctccaccatttttg

SEQ ID NO: 12 - DNA, 18 bp, Homo sapiens
tcaccgtccagcctccat

SEQ ID NO: 13 - DNA, 18 bp, Homo sapiens
caactgtgagatgacttc

SEQ ID NO: 14 - DNA, 17 bp, Homo sapiens
cgccacccgcttacaca

SEQ ID NO: 15 - DNA, 22 bp, Homo sapiens
cagaggctggatctggaaaagt

SEQ ID NO: 16 - DNA, 15 bp, Homo sapiens
tgccaggaactcttt

SEQ ID NO: 17 - DNA, 23 bp, Homo sapiens
tacaggctaccaccctgttgatc

SEQ ID NO: 18 - DNA, 17 bp, Homo sapiens
aaccgcgggccctctag

SEQ ID NO: 19 - DNA, 17 bp, Homo sapiens
ccatggaggctacagca

SEQ ID NO: 20 - DNA, 27 bp, Homo sapiens
cttgaagggattgaaaagataattagc

SEQ ID NO: 21 - DNA, 24 bp, Homo sapiens
ccatgagtcagaaaagcattgaac

SEQ ID NO: 22 - DNA, 17 bp, Homo sapiens
aggtgagcattttcctg